European Patent Specification EP 4 504 342 B1, published April 29, 2026. Title: Bifunctional peptide with mucoadhesive and virus binding properties. Applicant: Freie Universität Berlin. The sequence listing filed with the application follows.

SEQUENCE LISTING (63 sequences)

SEQ ID NO: 1 - protein, 59 aa, Homo sapiens
EEYVGLSANQCAVPAKDRVDCGYPHVTPKECNNRGCCFDSRIPGVPWCFKPLQEAEKTF

SEQ ID NO: 2 - protein, 23 aa, Homo sapiens
EEQAKTFLDKFNHEAEDLFYQSS

SEQ ID NO: 3 - protein, 31 aa, Homo sapiens
EEQAKTFLDKFNHEAEDLFYQSSGLGKGDFR

SEQ ID NO: 4 - protein, 31 aa, Homo sapiens
  CROSSLNK 4..8: note = Side chain cyclization between lysine 4 and aspartate 8.
EEQKKTFDDKFNHEAEDLFYQSSGLGKGDFR

SEQ ID NO: 5 - protein, 31 aa, Homo sapiens
  CROSSLNK 8..12: note = Side chain cyclization between lysine 8 and aspartate 12.
EEQAKTFKDKFDHEAEDLFYQSSGLGKGDFR

SEQ ID NO: 6 - protein, 31 aa, Homo sapiens
  CROSSLNK 11..15: note = Side chain cyclization between lysine 11 and aspartate 15.
EEQAKTFLDKKNHEDEDLFYQSSGLGKGDFR

SEQ ID NO: 7 - protein, 31 aa, Homo sapiens
  CROSSLNK 15..19: note = Side chain cyclization between lysine 15 and aspartate 19.
EEQAKTFLDKFNHEKEDLDYQSSGLGKGDFR

SEQ ID NO: 8 - protein, 31 aa, Homo sapiens
  CROSSLNK 18..22: note = Side chain cyclization between lysine 18 and aspartate 22.
EEQAKTFLDKFNHEAEDKFYQDSGLGKGDFR

SEQ ID NO: 9 - protein, 31 aa, Homo sapiens
  CROSSLNK 8..12: note = Side chain cyclization between lysine 8 and aspartate 12.
  CROSSLNK 18..22: note = Side chain cyclization between lysine 18 and aspartate 22.
EEQAKTFKDKFDHEAEDKFYQDSGLGKGDFR

SEQ ID NO: 10 - protein, 31 aa, Homo sapiens
  SITE 15: note = X is an alkenylated (R)-alanine residue.
  CROSSLNK 15..22: note = Cyclization between X15 and X22 via a 7-undecenyl residue.
  SITE 22: note = X is an alkenylated (S)-alanine residue.
EEQAKTFLDKFNHEXEDLFYQXSGLGKGDFR

SEQ ID NO: 11 - protein, 31 aa, Homo sapiens
  SITE 1: note = X is N-acetylglutamate.
  SITE 15: note = X is an alkenylated (R)-alanine residue.
  CROSSLNK 15..22: note = Cyclization between X15 and X22 via a 7-undecenyl residue.
  SITE 22: note = X is an alkenylated (S)-alanine residue.
XEQAKTFLDKFNHEXEDLFYQXSGLGKGDFR

SEQ ID NO: 12 - protein, 31 aa, Homo sapiens
  SITE 18: note = X is an alkenylated (S)-alanine residue.
  CROSSLNK 18..22: note = Cyclization between X18 and X22 via a 4-octenyl residue.
  SITE 22: note = X is an alkenylated (S)-alanine residue.
EEQAKTFLDKFNHEAEDXFYQXSGLGKGDFR

SEQ ID NO: 13 - protein, 31 aa, Homo sapiens
  SITE 1: note = X is N-acetylglutamate.
  SITE 18: note = X is an alkenylated (S)-alanine residue.
  CROSSLNK 18..22: note = Cyclization between X18 and X22 via a 4-octenyl residue.
  SITE 22: note = X is an alkenylated (S)-alanine residue.
XEQAKTFLDKFNHEAEDXFYQXSGLGKGDFR

SEQ ID NO: 14 - protein, 59 aa, Homo sapiens
EEYVGLSANQCAVPAKDRVDCGYPHVTPKECNNRGCCFDSRIPGVPWCFKPLQEAECTF

SEQ ID NO: 15 - protein, 24 aa, synthetic construct
  REGION 1..24: note = Mucin binding moiety precursor
  SITE 22: note = X is azidolysine.
CCFDSRIPGVPWCFKPLQEAEXTF

SEQ ID NO: 16 - protein, 35 aa, synthetic construct
  REGION 1..35: note = Mucin binding moiety precursor
  SITE 35: note = X is a glycin residue modified with an N-acylbenzimidazole.
EEYVGLSANQCAVPAKDRVDCGYPHVTPKECNNRX

SEQ ID NO: 17 - protein, 31 aa, synthetic construct
  REGION 1..31: note = Virus binding moiety precursor
  SITE 1: note = X is a glutamte residue carrying a linker comprising two subsequent units of 8-amino-3,6-dioxaoctanoic acid, followed by a 4-pentynoic acid unit.
XEQAKTFLDKFNHEAEDLFYQSSGLGKGDFR

SEQ ID NO: 18 - protein, 88 aa, synthetic construct
  REGION 1..88: note = Peptide comprising a mucin binding moiety and a virus binding moiety
  SITE 57: note = X is a lysine residue modified at its C-terminus with a threonine-phenylalanine dipeptide. X is bound through its side chain to a 10,19-dioxo-21-(1H-1,2,3-triazol-4-yl)-3,6,12,15-tetraoxa-9,18-diazahenicosanoic acid linker. The free carboxylic acid in the linker is attached to the N-terminus of glutamate 58.
EEYVGLSANQCAVPAKDRVDCGYPHVTPKECNNRGCCFDSRIPGVPWCFKPLQEAEXEEQAKTFLDKFNHEAEDLFYQSSGLGKGDFR

SEQ ID NO: 19 - protein, 93 aa, synthetic construct
GEEYVGLSANQCAVPAKDRVDCGYPHVTPKECNNRGCCFDSRIPGVPWCFKPLQEAEATFGTEEQAKTFLDKFNHEAEDLFYQSSGLGKGDFR

SEQ ID NO: 20 - protein, 84 aa, Homo sapiens
MATMENKVICALVLVSMLALGTLAEAQTETCTVAPRERQNCGFPGVTPSQCANKGCCFDDTVRGVPWCFYPNTIDVPPEEECEF

SEQ ID NO: 21 - protein, 129 aa, Homo sapiens
MGRRDAQLLAALLVLGLCALAGSEKPSPCQCSRLSPHNRTNCGFPGITSDQCFDNGCCFDSSVTGVPWCFHPLPKQESDQCVMEVSDRRNCGYPGISPEECASRKCCFSNFIFEVPWCFFPKSVEDCHY

SEQ ID NO: 22 - protein, 217 aa, Artocarpus heterophyllus
MAYSSLLSLSVLALLFSISSADTRKWFLANGINQNPIGIIEAAVGVSEDLLNLNGMEAKNDEQSGISQTVIVGPWGAKVSTSSNGKAFDDGAFTGIREINLSYNKETAIGDFQVVYDLNGSPYVGQNHKSFITGFTPVKISLDFPSEYIMEVSGYTGNVSGYVVVRSLTFKTNKKTYGPYGVTSGTPFNLPIENGLIVGFKGSIGYWLDYFSMYLSL

SEQ ID NO: 23 - protein, 23 aa, synthetic construct
ECQAKTFLDKFNHEAEDLFYQSS

SEQ ID NO: 24 - protein, 23 aa, synthetic construct
EECAKTFLDKFNHEAEDLFYQSS

SEQ ID NO: 25 - protein, 23 aa, synthetic construct
EEQCKTFLDKFNHEAEDLFYQSS

SEQ ID NO: 26 - protein, 23 aa, synthetic construct
EEQACTFLDKFNHEAEDLFYQSS

SEQ ID NO: 27 - protein, 23 aa, synthetic construct
EEQAKCFLDKFNHEAEDLFYQSS

SEQ ID NO: 28 - protein, 23 aa, synthetic construct
EEQAKTCLDKFNHEAEDLFYQSS

SEQ ID NO: 29 - protein, 23 aa, synthetic construct
EEQAKTFCDKFNHEAEDLFYQSS

SEQ ID NO: 30 - protein, 23 aa, synthetic construct
EEQAKTFLCKFNHEAEDLFYQSS

SEQ ID NO: 31 - protein, 23 aa, synthetic construct
EEQAKTFLDCFNHEAEDLFYQSS

SEQ ID NO: 32 - protein, 23 aa, synthetic construct
EEQAKTFLDKCNHEAEDLFYQSS

SEQ ID NO: 33 - protein, 23 aa, synthetic construct
EEQAKTFLDKFCHEAEDLFYQSS

SEQ ID NO: 34 - protein, 23 aa, synthetic construct
EEQAKTFLDKFNCEAEDLFYQSS

SEQ ID NO: 35 - protein, 23 aa, synthetic construct
EEQCKTFCDKFNHEAEDLFYQSS

SEQ ID NO: 36 - protein, 23 aa, synthetic construct
EEQAKTFCDKFCHEAEDLFYQSS

SEQ ID NO: 37 - protein, 23 aa, synthetic construct
EEQAKTFLDKCNHECEDLFYQSS

SEQ ID NO: 38 - protein, 23 aa, synthetic construct
EEQAKTFLDKFNHECEDLCYQSS

SEQ ID NO: 39 - protein, 23 aa, synthetic construct
EEQAKTFLDKFNHEAEDCFYQCS

SEQ ID NO: 40 - protein, 23 aa, synthetic construct
EEQCKTFCDKFNHEAEDCFYQCS

SEQ ID NO: 41 - protein, 36 aa, synthetic construct
EAAAKEEQAKTFLDKFNHEAEDLFYQSSGLGKGDFR

SEQ ID NO: 42 - protein, 32 aa, synthetic construct
  DISULFID 23..32: note = Disulfide bridge between cysteine 23 and cysteine 32.
EEQAKTFLDKFNHEAEDLFYQSCGLGKGDFRC

SEQ ID NO: 43 - protein, 37 aa, synthetic construct
  DISULFID 28..37: note = Disulfide bridge between cysteine 28 and cysteine 37.
EAAAKEEQAKTFLDKFNHEAEDLFYQSCGLGKGDFRC

SEQ ID NO: 44 - protein, 5 aa, synthetic construct
GGGGS

SEQ ID NO: 45 - protein, 5 aa, synthetic construct
EAAAK

SEQ ID NO: 46 - protein, 11 aa, synthetic construct
GTSGSGLPSTG

SEQ ID NO: 47 - protein, 10 aa, synthetic construct
GTSYAHQAHY

SEQ ID NO: 48 - protein, 15 aa, synthetic construct
ARDFYDYDVFYYAMD

SEQ ID NO: 49 - protein, 9 aa, synthetic construct
IQIIPKSSW

SEQ ID NO: 50 - protein, 9 aa, synthetic construct
RGHFYGSGS

SEQ ID NO: 51 - protein, 10 aa, synthetic construct
IQIIPKDSWS

SEQ ID NO: 52 - protein, 9 aa, synthetic construct
PTIKKGYNN

SEQ ID NO: 53 - protein, 14 aa, synthetic construct
CARLYTKSSNANYW

SEQ ID NO: 54 - protein, 15 aa, synthetic construct
CARGGLYSSDAFDVW

SEQ ID NO: 55 - protein, 49 aa, synthetic construct
KLLGIETPLPKKELLLPGNNRKVYELSNVQEDSQPMCYSNCPDGQSTAK

SEQ ID NO: 56 - protein, 11 aa, synthetic construct
RSGNYPYAMDY

SEQ ID NO: 57 - protein, 12 aa, synthetic construct
GLPDLEWLLYPN

SEQ ID NO: 58 - protein, 12 aa, synthetic construct
SISASGSYINYA

SEQ ID NO: 59 - protein, 12 aa, synthetic construct
RDGGRELSPFEK

SEQ ID NO: 60 - protein, 12 aa, synthetic construct
SISASGSYINYA

SEQ ID NO: 61 - protein, 14 aa, synthetic construct
LVVSTTYLPHYFDN

SEQ ID NO: 62 - protein, 14 aa, synthetic construct
LVVSETYLPHYFDN

SEQ ID NO: 63 - protein, 14 aa, synthetic construct
  SITE 1: note = X is L-cyclohexylglycine
  SITE 2: note = X is cyclopropylalanine
  SITE 7: note = X is 3,5-diiodo-tyrosine
XXVSTTXLPHYFDN